European Patent Application EP 4 427 763 A1, published September 11, 2024. Title: ANTITUMOR COMBINATIONS CONTAINING ANTI-CEACAM5 ANTIBODY-DRUG CONJUGATES, ANTI-VEGFR-2 ANTIBODIES AND ANTI-PD1/PD-L1 ANTIBODIES. Applicant: SANOFI. The sequence listing filed with the application follows.

SEQUENCE LISTING (17 sequences)

SEQ ID NO: 1 - protein, 8 aa, synthetic construct
  REGION 1..8: note = CDR-H1 of anti-CEACAM5-antibody
GFVFSSYD

SEQ ID NO: 2 - protein, 8 aa, synthetic construct
  REGION 1..8: note = CDR-H2 of anti-CEACAM5-antibody
ISSGGGIT

SEQ ID NO: 3 - protein, 13 aa, synthetic construct
  REGION 1..13: note = CDR-H3 of anti-CEACAM5-antibody
AAHYFGSSGPFAY

SEQ ID NO: 4 - protein, 6 aa, synthetic construct
  REGION 1..6: note = CDR-L1 of anti-CEACAM5-antibody
ENIFSY

SEQ ID NO: 5 - protein, 9 aa, synthetic construct
  REGION 1..9: note = CDR-L3 of anti-CEACAM5-antibody
QHHYGTPFT

SEQ ID NO: 6 - protein, 120 aa, synthetic construct [sequence omitted]

SEQ ID NO: 7 - protein, 107 aa, synthetic construct [sequence omitted]

SEQ ID NO: 8 - protein, 449 aa, synthetic construct
  REGION 1..449: note = Heavy chain of anti-CEACAM5-antibody
EVQLQESGPGLVKPGGSLSLSCAASGFVFSSYDMSWVRQTPERGLEWVAYISSGGGITYAPSTVKGRFTVSRDNAKNTLYLQMNSLTSEDTAVYYCAAHYFGSSGPFAYWGQGTLVTVSSASTKGPSVFPLAPSSKSTSGGTAALGCLVKDYFPEPVTVSWNSGALTSGVHTFPAVLQSSGLYSLSSVVTVPSSSLGTQTYICNVNHKPSNTKVDKKVEPKSCDKTHTCPPCPAPELLGGPSVFLFPPKPKDTLMISRTPEVTCVVVDVSHEDPEVKFNWYVDGVEVHNAKTKPREEQYNSTYRVVSVLTVLHQDWLNGKEYKCKVSNKALPAPIEKTISKAKGQPREPQVYTLPPSRDELTKNQVSLTCLVKGFYPSDIAVEWESNGQPENNYKTTPPVLDSDGSFFLYSKLTVDKSRWQQGNVFSCSVMHEALHNHYTQKSLSLSPG

SEQ ID NO: 9 - protein, 214 aa, synthetic construct
  REGION 1..214: note = Light chain of anti-CEACAM5-antibody
DIQMTQSPASLSASVGDRVTITCRASENIFSYLAWYQQKPGKSPKLLVYNTRTLAEGVPSRFSGSGSGTDFSLTISSLQPEDFATYYCQHHYGTPFTFGSGTKLEIKRTVAAPSVFIFPPSDEQLKSGTASVVCLLNNFYPREAKVQWKVDNALQSGNSQESVTEQDSKDSTYSLSSTLTLSKADYEKHKVYACEVTHQGLSSPVTKSFNRGEC

SEQ ID NO: 10 - protein, 446 aa, synthetic construct
  REGION 1..446: note = Heavy chain of Ramucirumab
EVQLVQSGGGLVKPGGSLRLSCAASGFTFSSYSMNWVRQAPGKGLEWVSSISSSSSYIYYADSVKGRFTISRDNAKNSLYLQMNSLRAEDTAVYYCARVTDAFDIWGQGTMVTVSSASTKGPSVLPLAPSSKSTSGGTAALGCLVKDYFPEPVTVSWNSGALTSGVHTFPAVLQSSGLYSLSSVVTVPSSSLGTQTYICNVNHKPSNTKVDKRVEPKSCDKTHTCPPCPAPELLGGPSVFLFPPKPKDTLMISRTPEVTCVVVDVSHEDPEVKFNWYVDGVEVHNAKTKPREEQYNSTYRVVSVLTVLHQDWLNGKEYKCKVSNKALPAPIEKTISKAKGQPREPQVYTLPPSREEMTKNQVSLTCLVKGFYPSDIAVEWESNGQPENNYKTTPPVLDSDGSFFLYSKLTVDKSRWQQGNVFSCSVMHEALHNHYTQKSLSLSPGK

SEQ ID NO: 11 - protein, 214 aa, synthetic construct
  REGION 1..214: note = Light chain of Ramucirumab
DIQMTQSPSSVSASIGDRVTITCRASQGIDNWLGWYQQKPGKAPKLLIYDASNLDTGVPSRFSGSGSGTYFTLTISSLQAEDFAVYFCQQAKAFPPTFGGGTKVDIKRTVAAPSVFIFPPSDEQLKSGTASVVCLLNNFYPREAKVQWKVDNALQSGNSQESVTEQDSKDSTYSLSSTLTLSKADYEKHKVYACEVTHQGLSSPVTKSFNRGEC

SEQ ID NO: 12 - protein, 10 aa, synthetic construct
  REGION 1..10: note = CDR-H1 of anti-VEGFR2-antibody
GFTFSSYSMN

SEQ ID NO: 13 - protein, 17 aa, synthetic construct
  REGION 1..17: note = CDR-H2 of anti-VEGFR2-antibody
SISSSSSYIYYADSVKG

SEQ ID NO: 14 - protein, 7 aa, synthetic construct
  REGION 1..7: note = CDR-H3 of anti-VEGFR2-antibody
VTDAFDI

SEQ ID NO: 15 - protein, 11 aa, synthetic construct
  REGION 1..11: note = CDR-L1 of anti-VEGFR2-antibody
RASQGIDNWLG

SEQ ID NO: 16 - protein, 7 aa, synthetic construct
  REGION 1..7: note = CDR-L2 of anti-VEGFR2-antibody
DASNLDT

SEQ ID NO: 17 - protein, 9 aa, synthetic construct
  REGION 1..9: note = CDR-L3 of anti-VEGFR2-antibody
QQAKAFPPT